European Patent Application EP 4 567 818 A1, published June 11, 2025. Title: METHOD FOR DESIGNING HUMANIZED ANTIBODY SEQUENCE. Applicant: Nanjing GenScript Biotech Co., Ltd. Application EP PCT/CN2023/117671, filed September 8, 2023. The sequence listing filed with the application follows.

SEQUENCE LISTING (29 sequences)

SEQ ID NO: 1 - protein, 255 aa, Homo sapiens
MGNSCYNIVATLLLVLNFERTRSLQDPCSNCPAGTFCDNNRNQICSPCPPNSFSSAGGQRTCDICRQCKGVFRTRKECSSTSNAECDCTPGFHCLGAGCSMCEQDCKQGQELTKKGCKDCCFGTFNDQKRGICRPWTNCSLDGKSVLVNGTKERDVVCGPSPADLSPGASSVTPPAPAREPGHSPQIISFFLALTSTALLFLLFFLTLRFSVVKRGRKKLLYIFKQPFMRPVQTTQEEDGCSCRFPEEEEGGCEL

SEQ ID NO: 2 - protein, 117 aa, Rabbit
QSVEESGGRLVTPGTPLTLTCTVSGFSLGTFPIGWVRQAPGSGLEWIGIFNTDGSAAYASWARGRFTVFKNSTTVDLKMTSPTTEDTATYFCARINADYSGWYFGIWGPGTLVTVSS

SEQ ID NO: 3 - protein, 13 aa, Rabbit
TVSGFSLGTFPIG

SEQ ID NO: 4 - protein, 9 aa, Rabbit
IFNTDGSAA

SEQ ID NO: 5 - protein, 14 aa, Rabbit
ARINADYSGWYFGI

SEQ ID NO: 6 - protein, 106 aa, Rabbit
EMTQTPASVEVAVGGTVTIKCQASQSIYSYLAWYQQKPGQPPKPLIYEASKTPSGVPSRFKGSGSGTEYTLTISGVQCEDAATYYCQKGYSVSNVAFGGGTEVVVK

SEQ ID NO: 7 - protein, 11 aa, Rabbit
QASQSIYSYLA

SEQ ID NO: 8 - protein, 8 aa, Rabbit
YEASKTPS

SEQ ID NO: 9 - protein, 10 aa, Rabbit
QKGYSVSNVA

SEQ ID NO: 10 - protein, 152 aa, synthetic construct
  UNSURE 2
  UNSURE 10
  UNSURE 31..34
  UNSURE 60..62
  UNSURE 73
  UNSURE 84..85
  UNSURE 112..134
QXSVEESGGXRLVTPGTPLTLTCTVSGFSLXXXXGTFPIGWVRQAPGSGLEWIGIFNTDXXXGSAAYASWARXGRFTVFKNSTXXTVDLKMTSPTTEDTATYFCARINADYXXXXXXXXXXXXXXXXXXXXXXXSGWYFGIWGPGTLVTVSS

SEQ ID NO: 11 - protein, 134 aa, synthetic construct
  UNSURE 1..2
  UNSURE 30..35
  UNSURE 58..64
  UNSURE 73
  UNSURE 81..82
  UNSURE 110..119
XXEMTQTPASVEVAVGGTVTIKCQASQSIXXXXXXYSYLAWYQQKPGQPPKPLIYEAXXXXXXXSKTPSGVPXSRFKGSGXXSGTEYTLTISGVQCEDAATYYCQKGYSXXXXXXXXXXVSNVAFGGGTEVVVK

SEQ ID NO: 12 - protein, 152 aa, Homo sapiens
  UNSURE 16
  UNSURE 37..40
  UNSURE 79
  UNSURE 122..137
EVQLVESGGXGLVQPGRSLRLSCTASGFTFXXXXGDYAMSWVRQAPGRGLEWIGFIRSKVYDGTTEYAASVKXGRFTISRDDSKSIAHLQMNSLTTEDTAVYYCSRLRADSSDYYXXXXXXXXXXXXXXXXSSPGSYYFDYWGQGTLVTVSS

SEQ ID NO: 13 - protein, 120 aa, synthetic construct
EVQLVESGGGLVQPGRSLRLSCTVSGFSLGTFPIGWVRQAPGRGLEWIGIFNTDGSAAYAASVKGRFTISRDDSKSIAHLQMNSLTTEDTAVYYCARINADYSGWYFGIWGQGTLVTVSS

SEQ ID NO: 14 - protein, 152 aa, synthetic construct
  UNSURE 2
  UNSURE 10
  UNSURE 24..40
  UNSURE 55..66
  UNSURE 73
  UNSURE 84..85
  UNSURE 105..141
QXSVEESGGXRLVTPGTPLTLTCXXXXXXXXXXXXXXXXXWVRQAPGSGLEWIGXXXXXXXXXXXXYASWARXGRFTVFKNSTXXTVDLKMTSPTTEDTATYFCXXXXXXXXXXXXXXXXXXXXXXXXXXXXXXXXXXXXXWGPGTLVTVSS

SEQ ID NO: 15 - protein, 152 aa, synthetic construct
  UNSURE 16
  UNSURE 37..40
  UNSURE 79
  UNSURE 117..142
EVQLEESGGXGLVQPGGSLKLSCAASGFTLXXXXSGSSMHWVRQAPGKGLEWVGRIRSKTNSNATAYAASVKXGRFTVSRDDSKNTVYLHMNSLKTEDTAVYFCTRTMTLXXXXXXXXXXXXXXXXXXXXXXXXXXAAFDYWGQGTLVTVSS

SEQ ID NO: 16 - protein, 120 aa, synthetic construct
EVQLEESGGGLVQPGGSLKLSCTVSGFSLGTFPIGWVRQAPGKGLEWVGIFNTDGSAAYAASVKGRFTVSRDDSKNTVYLHMNSLKTEDTAVYFCARINADYSGWYFGIWGQGTLVTVSS

SEQ ID NO: 17 - protein, 134 aa, synthetic construct
  UNSURE 36..41
  UNSURE 64..70
  UNSURE 79
  UNSURE 87..88
  UNSURE 115..126
DIQMTQSPSSLSVSVGGRVTITCRASQSIXXXXXXSSYLNWYQQKPGKAPKLLIYAAXXXXXXXSSLQSGVPXSRFNGNGXXSGTDFTLTISSLQPEDSATYYCQQSYXXXXXXXXXXXXSILLFGGGTEVEIK

SEQ ID NO: 18 - protein, 108 aa, synthetic construct
DIQMTQSPSSLSVSVGGRVTITCQASQSIYSYLAWYQQKPGKAPKLLIYEASKTPSGVPSRFNGNGSGTDFTLTISSLQPEDSATYYCQKGYSVSNVAFGGGTEVEIK

SEQ ID NO: 19 - protein, 134 aa, synthetic construct
  UNSURE 1..2
  UNSURE 24..40
  UNSURE 55..69
  UNSURE 73
  UNSURE 81..82
  UNSURE 105..124
XXEMTQTPASVEVAVGGTVTIKCXXXXXXXXXXXXXXXXXWYQQKPGQPPKPLIXXXXXXXXXXXXXXXGVPXSRFKGSGXXSGTEYTLTISGVQCEDAATYYCXXXXXXXXXXXXXXXXXXXXFGGGTEVVVK

SEQ ID NO: 20 - protein, 120 aa, synthetic construct
EVQLEESGGGLVQPGGSLALSCTVSGFSLGTFPIGWVRQAPGKGLEWVGIFNTDGSAAYAASVKGRFTVSRDSSKNTFYLHMNSLKTEDTAVYFCARINADYSGWYFGIWGQGTLVDVSS

SEQ ID NO: 21 - protein, 120 aa, synthetic construct
EVQLEESGGGLVQPGMSLRLSCTVSGFSLGTFPIGWVRQAPGKGLEWVGIFNTDGSAAYAASVKGRFNVSKNSTKNTVYLHMNSLKTEDTAVYFCARINADYSGWYFGIWGQGTLVTVSS

SEQ ID NO: 22 - protein, 120 aa, synthetic construct
EVQLEESGGGLVQPGGSLALSCTVSGFSLGTFPIGWVRQAPGKGLEWVGIFNTDGSAAYAASVKGRFTVSRDSSKNTVYLHMNSLKTEDTAVYFCARINADYSGWYFGIWGQGTLVTVSS

SEQ ID NO: 23 - protein, 120 aa, synthetic construct
EVQLEESGGGVVQPGGSLKLSCTVSGFSLGTFPIGWVRQAPGKGLEWVGIFNTDGSAAYAASVKGRFTVSKNSTKNTVYLHMNSLKTEDTAVYFCARINADYSGWYFGIWGQGTLVTVSS

SEQ ID NO: 24 - protein, 108 aa, synthetic construct
AQQMTQSPSSLSVSVGGRVTITCQASQSIYSYLAWYQQKPGKAPKLLIYEASKTPSGVPSRFNGNGSGTEYTLTISSLQPEDSATYYCQKGYSVSNVAFGGGTEVEIK

SEQ ID NO: 25 - protein, 108 aa, synthetic construct
DIQMTQSPSSLSASVGGRVTITCQASQSIYSYLAWYQQKPGKAPKLLIYEASKTPSGVPSRFNGNGSGTDFTLTISSLQPEDSATYYCQKGYSVSNVAFGGGTEVEIK

SEQ ID NO: 26 - protein, 108 aa, synthetic construct
DIQMTQSPSSLSVSVGGRVTITCQASQSIYSYLAWYQQKPGKAPKLLIYEASKTPSGVPSRFNGNGSGTEYTLTISSLQPEDSATYYCQKGYSVSNVAFGGGTEVEIK

SEQ ID NO: 27 - protein, 330 aa, synthetic construct [sequence omitted]

SEQ ID NO: 28 - protein, 107 aa, synthetic construct [sequence omitted]

SEQ ID NO: 29 - protein, 19 aa, Homo sapiens
MGWSCIILFLVATATGVHS